European Patent Application EP 4 442 832 A2, published October 9, 2024. Title: MICROBIAL COMPOSITIONS COMPRISING ELLAGITANNIN AND METHODS OF USE. Applicant: MARVELBIOME, INC. Application AU 2023285750, filed December 19, 2023. The sequence listing filed with the application follows.

SEQUENCE LISTING (9 sequences)

SEQ ID NO: 1 - DNA, 1410 bp, Lactobacillus plantarum
  source 1..1410: mol_type = unassigned DNA
atgagtaaccgattgatttttgatgctgactggctggtgccggaacaggtccaagttgccgggcaggctattcaatattatgctgcccgtaatattcagtacgttcagcatccagtcgcagcgattcaggtcctaaacgtttttgtaccagccgcatacttgcatggcagttcagtcaatggttatcagcgggcaacggcgccaattctgatgccgaatacggtcggcggttatttgccaggaccggcggatgatccgcaacgtgtcacttggccgacgaatgcagggacgattcaacaggcacttaaacgcggttacgttgtggtggccgctggaattcgcggtcgtacgacggttgataagtctgggcaacgggtcgggcaagcgccggcttttatcgtagatatgaaggcggcaatccgttacgttaagtataatcagggccggctgccaggtgacacgaaccggatcatcacgaatggaacgagtgctgggggtgccacttcggctttagcgggtgcgagtggcaattcggcttattttgaaccagccttaactgcgctcggggcagcaccggcgactgacgatatctttgcggtgtcagcttactgcccgattcataatctggaacacgcagacatggcctacgagtggcagtttaatggtattaatgactggcaccgttatcagcctgttgcggggacgaccaagaatgggcgaccaaaatttgaaccggttagtggtcagctcacagttgaagaacaggccctttcgttggcgttaaaagcccagttcagtacctacttgaaccagttgaaactcacggccagtgacgggacgcacttgacgcttaatgaggcgggaatgggttcatttcgtgatgttgttcgccaattattgatatcatctgctcagacggcattcgatcaagggacggatattcataagtacgcaggctttgtcgttactggaaatcaggtgacggacttggatttatcagcttatttgaagtcgttaactcgcatgaaagccgtcccggcgtttgaccaattagatttgacgagtccagagaataatttgtttggcgatgcaacggcgaaagccaagcactttacggccttggcacagacgcgaagtacggtgacggcacaactagcggacgctgagctgattcaggcgattaatccgctcagttacttaacgacaacttcgtcacgagttgctaagcactggcggattcgccacggtgcggccgaccgagatacgagttttgcaatcccgattattctagcaataatgttagaaaatcatggttatggcattgattttgcgctaccgtgggatattccccacagtggtgactatgatttaggcgatttattttcctggattgatggcttgtgccaatga

SEQ ID NO: 2 - protein, 469 aa, Lactobacillus plantarum
MSNRLIFDADWLVPEQVQVAGQAIQYYAARNIQYVQHPVAAIQVLNVFVPAAYLHGSSVNGYQRATAPILMPNTVGGYLPGPADDPQRVTWPTNAGTIQQALKRGYVVVAAGIRGRTTVDKSGQRVGQAPAFIVDMKAAIRYVKYNQGRLPGDTNRIITNGTSAGGATSALAGASGNSAYFEPALTALGAAPATDDIFAVSAYCPIHNLEHADMAYEWQFNGINDWHRYQPVAGTTKNGRPKFEPVSGQLTVEEQALSLALKAQFSTYLNQLKLTASDGTHLTLNEAGMGSFRDVVRQLLISSAQTAFDQGTDIHKYAGFVVTGNQVTDLDLSAYLKSLTRMKAVPAFDQLDLTSPENNLFGDATAKAKHFTALAQTRSTVTAQLADAELIQAINPLSYLTTTSSRVAKHWRIRHGAADRDTSFAIPIILAIMLENHGYGIDFALPWDIPHSGDYDLGDLFSWIDGLCQ

SEQ ID NO: 3 - DNA, 1473 bp, Lactobacillus plantarum
  source 1..1473: mol_type = unassigned DNA
atggcagaacaaccatgggatttgcgtcgcgtgcttgatgagatcaaggatgatccaaagaactatcatgaaactgacgtcgaagttgatccaaatgcggaactttctggtgtttatcggtatatcggtgctggtgggaccgttcaacggccaacgcaagagggtccagcaatgatgtttaacaacgttaaggggtttcctgatacgcgggtcttgactggattgatggcgagtcgccggcgcgttggtaagatgttccaccacgattatcagacgttagggcaatacttgaacgaagcagtctctaatccagtggcgccagaaacggttgctgaagcggatgcgccagctcacgatgtcgtttataaagcgacggatgaaggctttgatattcgtaagttagtggcagcaccaacgaatacgccccaagatgctggaccatatattacggtcggtgtggtgtttggctcaagcatggacaagtctaagagtgatgtgacgattcaccgaatggtccttgaagataaggataagttagggatttatatcatgcctggcggtcggcacattggtgcgtttgcggaagagtatgagaaagctaacaagccaatgccaattacaattaatattggtttggatccagccattacgattggtgcaactttcgaaccaccgaccacgccattcggttataacgaattaggtgttgctggtgcgattcggaaccaagctgttcaattagttgacggggtgaccgtcgatgaaaaggcgattgcgcgttctgaatatacgcttgaggggtacattatgcctaacgaacgtattcaggaagatatcaatacgcatacgggcaaggcgatgcctgaattcccgggttatgatggtgacgccaacccagctttacaagtgattaaggtgacggcggtgactcatcggaagaatgccatcatgcaaagcgtgattggaccatccgaagaacatgtcagcatggcgggaattccaactgaagctagtatcttacaattggttaaccgtgccattcctggtaaagtgacgaatgtttataatccgccggctggtggtggtaagttgatgaccatcatgcagattcacaaggataatgaagcggatgaaggaattcaacggcaagctgccttgcttgcgttctcagcctttaaggaattgaagactgttatcctggttgatgaagatgttgatatttttgatatgaatgatgtgatttggacgatgaatacccgtttccaagccgatcaggacttgatggtcttatcaggcatgcggaatcatccgttggacccatcggaacgcccacaatatgatccaaagtcgattcgtttccgtgggatgagttctaaactagtgattgatggcaccgtaccattcgatatgaaggaccaatttgaacgggcccaattcatgaaagtggctgactgggagaagtatttgaagtaa

SEQ ID NO: 4 - protein, 490 aa, Lactobacillus plantarum
MAEQPWDLRRVLDEIKDDPKNYHETDVEVDPNAELSGVYRYIGAGGTVQRPTQEGPAMMFNNVKGFPDTRVLTGLMASRRRVGKMFHHDYQTLGQYLNEAVSNPVAPETVAEADAPAHDVVYKATDEGFDIRKLVAAPTNTPQDAGPYITVGVVFGSSMDKSKSDVTIHRMVLEDKDKLGIYIMPGGRHIGAFAEEYEKANKPMPITINIGLDPAITIGATFEPPTTPFGYNELGVAGAIRNQAVQLVDGVTVDEKAIARSEYTLEGYIMPNERIQEDINTHTGKAMPEFPGYDGDANPALQVIKVTAVTHRKNAIMQSVIGPSEEHVSMAGIPTEASILQLVNRAIPGKVTNVYNPPAGGGKLMTIMQIHKDNEADEGIQRQAALLAFSAFKELKTVILVDEDVDIFDMNDVIWTMNTRFQADQDLMVLSGMRNHPLDPSERPQYDPKSIRFRGMSSKLVIDGTVPFDMKDQFERAQFMKVADWEKYLK

SEQ ID NO: 5 - DNA, 564 bp, Lactobacillus plantarum
  source 1..564: mol_type = unassigned DNA
atgaaacgaattgttgtgggaatcacgggagcgtccggtacgatttacgcggtcgacttattagaaaagttacatcagcggccagatgttgaagttcatctggtaatgagtgcgtgggctaaaaaaaacttggagttagagactgattactcgctcgcgcagctgacggcgctcgcggatgctacttatcgggctaatgaccaaggcgcagcgattgccagcggttcgtttttgaatgacggaatggtcattgtcccagctagtatgaagacggtagcagggattgcgtacggcttcggtgataatttaatatcgcgggctgctgatgtcacgattaaagaacaacgtaaacttgtgattgttccacgtgaaacaccgttaagcgtgattcatttagaaaatctaacgaagttggcaaaactcggtgcccaaattattccaccgattcccgcgttttataatcatccgcaatccattcaggatctggtcaatcatcaaaccatgaaaattttagatgcgtttcatattcataatgaaactgatcgccgttgggagggggattaa

SEQ ID NO: 6 - protein, 187 aa, Lactobacillus plantarum
MKRIVVGITGASGTIYAVDLLEKLHQRPDVEVHLVMSAWAKKNLELETDYSLAQLTALADATYRANDQGAAIASGSFLNDGMVIVPASMKTVAGIAYGFGDNLISRAADVTIKEQRKLVIVPRETPLSVIHLENLTKLAKLGAQIIPPIPAFYNHPQSIQDLVNHQTMKILDAFHIHNETDRRWEGD

SEQ ID NO: 7 - DNA, 411 bp, Lactobacillus plantarum
  source 1..411: mol_type = unassigned DNA
atggcaacttttacgactgagcaggccgggtatcaaatgcaagcaatactccaagtgattggatatgacttgttgatcgtcgttaccggtgggaccaatccccatattggtgacgtgaccacactaactgccagcacggttcccgaaacggttaagtttcccagccatgatggtcgcttccacaaagataactttatttcggaacgaatggccaagcggattcagcgttatctagctggaagctgtacaattactgcgggaattcatgtcaaccaaattactaaagcacaaatagcagctgcggcaccaatgacggatgacctcagccgccagattattagctggttacaggcccatcccgtccaggctgaaaagccggaatattatggacaagacgagcaaccgcggtag

SEQ ID NO: 8 - protein, 136 aa, Lactobacillus plantarum
MATFTTEQAGYQMQAILQVIGYDLLIVVTGGTNPHIGDVTTLTASTVPETVKFPSHDGRFHKDNFISERMAKRIQRYLAGSCTITAGIHVNQITKAQIAAAAPMTDDLSRQIISWLQAHPVQAEKPEYYGQDEQPR

SEQ ID NO: 9 - protein, 40 aa, synthetic construct
  REGION 1..40: note = Description of Artificial Sequence: Synthetic polypeptide
QQQQQQQQQQQQQQQQQQQQQQQQQQQQQQQQQQQQQQQQ